European Patent Specification EP 3 916 009 B1, published June 28, 2023. Title: Recombinant proteins based on fibrinogen. Applicant: Sartorius Lab Instruments GmbH & Co. KG. The sequence listing filed with the application follows.

SEQUENCE LISTING (11 sequences)

SEQ ID NO: 1 - protein, 412 aa, Artificial sequence
  Fibrinogen gamma chain (FGG)
MYVATRDNCCILDERFGSYCPTTCGIADFLSTYQTKVDKDLQSLEDILHQVENKTSEVKQLIKAIQLTYNPDESSKPNMIDAATLKSRKMLEEIMKYEASILTHDSSIRYLQEIYNSNNQKIVNLKEKVAQLEAQCQEPCKDTVQIHDITGKDCQDIANKGAKQSGLYFIKPLKANQQFLVYCEIDGSGNGWTVFQKRLDGSVDFKKNWIQYKEGFGHLSPTGTTEFWLGNEKIHLISTQSAIPYALRVELEDWNGRTSTADYAMFKVGPEADKYRLTYAYFAGGDAGDAFDGFDFGDDPSDKFFTSHNGMQFSTWDNDNDKFEGNCAEQDGSGWWMNKCHAGHLNGVYYQGGTYSKASTPNGYDNGIIWATWKTRWYSMKKTTMKIIPFNRLTIGEGQQHHLGGAKQAGDV

SEQ ID NO: 2 - protein, 26 aa, Artificial sequence
  His-Tag
MGHHHHHHHHHHSSGHIEGRHMLEDI

SEQ ID NO: 3 - protein, 438 aa, Artificial sequence
  His-Tag-FGG
MGHHHHHHHHHHSSGHIEGRHMLEDIMYVATRDNCCILDERFGSYCPTTCGIADFLSTYQTKVDKDLQSLEDILHQVENKTSEVKQLIKAIQLTYNPDESSKPNMIDAATLKSRKMLEEIMKYEASILTHDSSIRYLQEIYNSNNQKIVNLKEKVAQLEAQCQEPCKDTVQIHDITGKDCQDIANKGAKQSGLYFIKPLKANQQFLVYCEIDGSGNGWTVFQKRLDGSVDFKKNWIQYKEGFGHLSPTGTTEFWLGNEKIHLISTQSAIPYALRVELEDWNGRTSTADYAMFKVGPEADKYRLTYAYFAGGDAGDAFDGFDFGDDPSDKFFTSHNGMQFSTWDNDNDKFEGNCAEQDGSGWWMNKCHAGHLNGVYYQGGTYSKASTPNGYDNGIIWATWKTRWYSMKKTTMKIIPFNRLTIGEGQQHHLGGAKQAGDV

SEQ ID NO: 4 - DNA, 1236 bp, Artificial sequence
  FGG coding sequence
atgtatgttgcaacccgtgataattgctgcattctggatgaacgttttggtagctattgtccgaccacctgtggtattgcagattttctgagcacctatcagaccaaagttgataaagatctgcagagcctggaagatattctgcatcaggttgaaaacaaaaccagcgaagttaaacagctgattaaagcaattcagctgacctataatccggatgaaagcagcaaaccgaatatgattgatgcagcaaccctgaaaagccgtaaaatgctggaagagatcatgaaatatgaagccagcattctgacccatgatagcagcattcgttatctgcaagaaatctacaatagcaataatcagaaaattgtgaatctgaaagaaaaagtggcacagctggaagcacagtgtcaagaaccgtgtaaagataccgttcagattcatgatatcaccggtaaagattgtcaggatattgcaaacaaaggtgcaaaacagagcggtctgtattttatcaaaccgctgaaagcaaatcagcagtttctggtgtattgcgaaattgatggtagcggtaatggttggaccgtttttcagaaacgtctggatggtagcgtggacttcaaaaaaaactggattcagtataaagaaggctttggtcatctgagcccgaccggcaccaccgaattttggctgggtaatgaaaaaattcatctgattagcacccagagcgcaattccgtatgcactgcgtgttgaactggaagattggaatggtcgtaccagcaccgcagattatgcaatgtttaaagttggtccggaagccgataaatatcgtctgacctatgcatattttgccggtggtgatgccggtgatgcatttgatggttttgattttggtgatgatccgagcgataaattctttaccagccataatggtatgcagtttagcacctgggataacgataacgataaatttgaaggcaattgtgccgaacaggatggtagtggttggtggatgaataaatgtcatgcaggtcatctgaacggcgtttattatcagggtggcacctatagcaaagcaagcaccccgaatggttatgataatggtattatttgggcaacctggaaaacccgttggtacagcatgaaaaaaaccaccatgaaaatcatcccgtttaaccgtctgaccattggtgaaggtcagcagcatcatctgggtggtgcaaaacaagccggtgatgtg

SEQ ID NO: 5 - DNA, 1268 bp, Artificial sequence
  Nucleic acid for FGG expression in E. coli
ctcgaggatatcatgtatgttgcaacccgtgataattgctgcattctggatgaacgttttggtagctattgtccgaccacctgtggtattgcagattttctgagcacctatcagaccaaagttgataaagatctgcagagcctggaagatattctgcatcaggttgaaaacaaaaccagcgaagttaaacagctgattaaagcaattcagctgacctataatccggatgaaagcagcaaaccgaatatgattgatgcagcaaccctgaaaagccgtaaaatgctggaagagatcatgaaatatgaagccagcattctgacccatgatagcagcattcgttatctgcaagaaatctacaatagcaataatcagaaaattgtgaatctgaaagaaaaagtggcacagctggaagcacagtgtcaagaaccgtgtaaagataccgttcagattcatgatatcaccggtaaagattgtcaggatattgcaaacaaaggtgcaaaacagagcggtctgtattttatcaaaccgctgaaagcaaatcagcagtttctggtgtattgcgaaattgatggtagcggtaatggttggaccgtttttcagaaacgtctggatggtagcgtggacttcaaaaaaaactggattcagtataaagaaggctttggtcatctgagcccgaccggcaccaccgaattttggctgggtaatgaaaaaattcatctgattagcacccagagcgcaattccgtatgcactgcgtgttgaactggaagattggaatggtcgtaccagcaccgcagattatgcaatgtttaaagttggtccggaagccgataaatatcgtctgacctatgcatattttgccggtggtgatgccggtgatgcatttgatggttttgattttggtgatgatccgagcgataaattctttaccagccataatggtatgcagtttagcacctgggataacgataacgataaatttgaaggcaattgtgccgaacaggatggtagtggttggtggatgaataaatgtcatgcaggtcatctgaacggcgtttattatcagggtggcacctatagcaaagcaagcaccccgaatggttatgataatggtattatttgggcaacctggaaaacccgttggtacagcatgaaaaaaaccaccatgaaaatcatcccgtttaaccgtctgaccattggtgaaggtcagcagcatcatctgggtggtgcaaaacaagccggtgatgtgtaataaaaggatccgtcgac

SEQ ID NO: 6 - DNA, 1334 bp, Artificial Sequence
  His-Tag-FGG coding sequence
atgggccatcatcatcatcatcatcatcatcatcacagcagcggccatatcgaaggtcgtcatatgctcgaggatatcatgtatgttgcaacccgtgataattgctgcattctggatgaacgttttggtagctattgtccgaccacctgtggtattgcagattttctgagcacctatcagaccaaagttgataaagatctgcagagcctggaagatattctgcatcaggttgaaaacaaaaccagcgaagttaaacagctgattaaagcaattcagctgacctataatccggatgaaagcagcaaaccgaatatgattgatgcagcaaccctgaaaagccgtaaaatgctggaagagatcatgaaatatgaagccagcattctgacccatgatagcagcattcgttatctgcaagaaatctacaatagcaataatcagaaaattgtgaatctgaaagaaaaagtggcacagctggaagcacagtgtcaagaaccgtgtaaagataccgttcagattcatgatatcaccggtaaagattgtcaggatattgcaaacaaaggtgcaaaacagagcggtctgtattttatcaaaccgctgaaagcaaatcagcagtttctggtgtattgcgaaattgatggtagcggtaatggttggaccgtttttcagaaacgtctggatggtagcgtggacttcaaaaaaaactggattcagtataaagaaggctttggtcatctgagcccgaccggcaccaccgaattttggctgggtaatgaaaaaattcatctgattagcacccagagcgcaattccgtatgcactgcgtgttgaactggaagattggaatggtcgtaccagcaccgcagattatgcaatgtttaaagttggtccggaagccgataaatatcgtctgacctatgcatattttgccggtggtgatgccggtgatgcatttgatggttttgattttggtgatgatccgagcgataaattctttaccagccataatggtatgcagtttagcacctgggataacgataacgataaatttgaaggcaattgtgccgaacaggatggtagtggttggtggatgaataaatgtcatgcaggtcatctgaacggcgtttattatcagggtggcacctatagcaaagcaagcaccccgaatggttatgataatggtattatttgggcaacctggaaaacccgttggtacagcatgaaaaaaaccaccatgaaaatcatcccgtttaaccgtctgaccattggtgaaggtcagcagcatcatctgggtggtgcaaaacaagccggtgatgtgtaataaaaggatccgtcgac

SEQ ID NO: 7 - protein, 4 aa, Artificial sequence
  Binding site
AGDV

SEQ ID NO: 8 - protein, 12 aa, Artificial Sequence
  Binding site on FGG
HHLGGAKQAGDV

SEQ ID NO: 9 - protein, 19 aa, Artificial Sequence
  Binding site on FGG
YSMKKTTMKIIPFNRLTIG

SEQ ID NO: 10 - protein, 12 aa, Artificial Sequence
  Binding site on FGG
WTVFQKRLDGSV

SEQ ID NO: 11 - protein, 13 aa, Artificial Sequence
  Binding site on FGG
GVYYQGGTYSKAS